European Patent Specification EP 3 831 844 B1, published March 13, 2024. Title: Diagnosis and therapy of Multiple Sclerosis. Applicant: Prindex S.r.l Paternò, R Avvedimento, VE Santillo, M Pavone, LM. The sequence listing filed with the application follows.

SEQUENCE LISTING (173 sequences)

SEQ ID NO: 1 - protein, 570 aa, Homo sapiens
MGNWAVNEGLSIFVILVWLGLNVFLFVWYYRVYDIPPKFFYTRKLLGSALALARAPAACLNFNCMLILLPVCRNLLSFLRGSSACCSTRVRRQLDRNLTFHKMVAWMIALHSAIHTIAHLFNVEWCVNARVNNSDPYSVALSELGDRQNESYLNFARKRIKNPEGGLYLAVTLLAGITGVVITLCLILIITSSTKTIRRSYFEVFWYTHHLFVIFFIGLAIHGAERIVRGQTAESLAVHNITVCEQKISEWGKIKECPIPQFAGNPPMTWKWIVGPMFLYLCERLVRFWRSQQKVVITKVVTHPFKTIELQMKKKGFKMEVGQYIFVKCPKVSKLEWHPFTLTSAPEEDFFSIHIRIVGDWTEGLFNACGCDKQEFQDAWKLPKIAVDGPFGTASEDVFSYEVVMLVGAGIGVTPFASILKSVWYKYCNNATNLKLKKIYFYWLCRDTHAFEWFADLLQLLESQMQERNNAGFLSYNIYLTGWDESQANHFAVHHDEEKDVITGLKQKTLYGRPNWDNEFKTIASQHPNTRIGVFLCGPEALAETLSKQSISNSESGPRGVHFIFNKENF

SEQ ID NO: 2 - protein, 471 aa, Homo sapiens
MDILCEENTSLSSTTNSLMQLNDDTRLYSNDFNSGEANTSDAFNWTVDSENRTNLSCEGCLSPSCLSLLHLQEKNWSALLTAVVIILTIAGNILVIMAVSLEKKLQNATNYFLMSLAIADMLLGFLVMPVSMLTILYGYRWPLPSKLCAVWIYLDVLFSTASIMHLCAISLDRYVAIQNPIHHSRFNSRTKAFLKIIAVWTISVGISMPIPVFGLQDDSKVFKEGSCLLADDNFVLIGSFVSFFIPLTIMVITYFLTIKSLQKEATLCVSDLGTRAKLASFSFLPQSSLSSEKLFQRSIHREPGSYTGRRTMQSISNEQKACKVLGIVFFLFVVMWCPFFITNIMAVICKESCNEDVIGALLNVFVWIGYLSSAVNPLVYTLFNKTYRSAFSRYIQCQYKENKKPLQLILVNTIPALAYKSSQLQMGQKKNSKQDAKTTDNDCSMVALGKQHSEEASKDNSDGVNEKVSCV

SEQ ID NO: 3 - protein, 19 aa, Homo sapiens
YRVYDIPPKFFYTRKLLGS

SEQ ID NO: 4 - protein, 46 aa, Homo sapiens
EWCVNARVNNSDPYSVALSELGDRQNESYLNFARKRIKNPEGGLYL

SEQ ID NO: 5 - protein, 40 aa, Homo sapiens
HGAERIVRGQTAESLAVHNITVCEQKISEWGKIKECPIPQ

SEQ ID NO: 6 - protein, 76 aa, Homo sapiens
MDILCEENTSLSSTTNSLMQLNDDTRLYSNDFNSGEANTSDAFNWTVDSENRTNLSCEGCLSPSCLSLLHLQEKNW

SEQ ID NO: 7 - protein, 16 aa, Homo sapiens
LTILYGYRWPLPSKLC

SEQ ID NO: 8 - protein, 19 aa, Homo sapiens
LQDDSKVFKEGSCLLADDN

SEQ ID NO: 9 - protein, 16 aa, Homo sapiens
VICKESCNEDVIGALL

SEQ ID NO: 10 - protein, 29 aa, Artificial Sequence
  synthetic
CNSLMQLNDDTRLYCMDILSEENTSLSSC

SEQ ID NO: 11 - protein, 29 aa, Artificial Sequence
  synthetic
CLTILYGYRWPLPSCMDILSEENTSLSSC

SEQ ID NO: 12 - protein, 15 aa, Artificial Sequence
  synthetic
LTILYGYRWPAASKL

SEQ ID NO: 13 - protein, 29 aa, Artificial Sequence
  synthetic
CLYGYRWPLPSKLSCMDILSEENTSLSSC

SEQ ID NO: 14 - protein, 9 aa, Artificial Sequence
  synthetic
YRWPLPSKL

SEQ ID NO: 15 - protein, 29 aa, Artificial Sequence
  synthetic
CNSLMQLNDDTRLYCLSSEGSLSPSSLSC

SEQ ID NO: 16 - protein, 29 aa, Artificial Sequence
  synthetic
CLQDDSKVFKEGSSCMDILSEENTSLSSC

SEQ ID NO: 17 - protein, 15 aa, Artificial Sequence
  synthetic
LTILYGYRWPLPSKL

SEQ ID NO: 18 - protein, 29 aa, Artificial Sequence
  synthetic
CMQLNDDTRLYSNDCMDILSEENTSLSSC

SEQ ID NO: 19 - protein, 29 aa, Artificial Sequence
  synthetic
CLSPSSLSLLHLQECMDILSEENTSLSSC

SEQ ID NO: 20 - protein, 29 aa, Artificial Sequence
  synthetic
CSTTNSLMQLNDDTCMDILSEENTSLSSC

SEQ ID NO: 21 - protein, 29 aa, Artificial Sequence
  synthetic
CLTILYGYRWPLPSCKESSNEDVIGALLC

SEQ ID NO: 22 - protein, 29 aa, Artificial Sequence
  synthetic
CTVDSENRTNLSSECMDILSEENTSLSSC

SEQ ID NO: 23 - protein, 9 aa, Artificial Sequence
  synthetic
GYRWPLPSK

SEQ ID NO: 24 - protein, 29 aa, Artificial Sequence
  synthetic
CMQLNDDTRLYSNDCSGEANTSDAFNWTC

SEQ ID NO: 25 - protein, 29 aa, Artificial Sequence
  synthetic
CDSKVFKEGSSLLACKESSNEDVIGALLC

SEQ ID NO: 26 - protein, 29 aa, Artificial Sequence
  synthetic
CENTSLSSTTNSLMCMDILSEENTSLSSC

SEQ ID NO: 27 - protein, 29 aa, Artificial Sequence
  synthetic
CSLSSTTNSLMQLNCMDILSEENTSLSSC

SEQ ID NO: 28 - protein, 29 aa, Artificial Sequence
  synthetic
CSLSSTTNSLMQLNCMDILSEENTSLSSC

SEQ ID NO: 29 - protein, 29 aa, Artificial Sequence
  synthetic
CLYGYRWPLPSKLSCKESSNEDVIGALLC

SEQ ID NO: 30 - protein, 29 aa, Artificial Sequence
  synthetic
CMDILSEENTSLSSCMQLNDDTRLYSNDC

SEQ ID NO: 31 - protein, 29 aa, Artificial Sequence
  synthetic
CSDAFNWTVDSENRCMDILSEENTSLSSC

SEQ ID NO: 32 - protein, 15 aa, Artificial Sequence
  synthetic
TVDSENRTNLAAEGC

SEQ ID NO: 33 - protein, 29 aa, Artificial Sequence
  synthetic
CNDDTRLYSNDFNSCMDILSEENTSLSSC

SEQ ID NO: 34 - protein, 29 aa, Artificial Sequence
  synthetic
CTVDSENRTNLSSECRTNLSSEGSLSPSC

SEQ ID NO: 35 - protein, 29 aa, Artificial Sequence
  synthetic
CLSSEGSLSPSSLSCMDILSEENTSLSSC

SEQ ID NO: 36 - protein, 29 aa, Artificial Sequence
  synthetic
CLSPSSLSLLHLQECTVDSENRTNLSSEC

SEQ ID NO: 37 - protein, 29 aa, Artificial Sequence
  synthetic
CDSKVFKEGSSLLACMDILSEENTSLSSC

SEQ ID NO: 38 - protein, 15 aa, Artificial Sequence
  synthetic
TILYGYRWPLPSKLC

SEQ ID NO: 39 - protein, 29 aa, Artificial Sequence
  synthetic
CFNWTVDSENRTNLCMDILSEENTSLSSC

SEQ ID NO: 40 - protein, 15 aa, Artificial Sequence
  synthetic
STTNSLMQLNAATRL

SEQ ID NO: 41 - protein, 29 aa, Artificial Sequence
  synthetic
CLYGYRWPLPSKLSCYSNDFNSGEANTSC

SEQ ID NO: 42 - protein, 15 aa, Artificial Sequence
  synthetic
QDDSKVFKEGAALLA

SEQ ID NO: 43 - protein, 29 aa, Artificial Sequence
  synthetic
CNSLMQLNDDTRLYCYSNDFNSGEANTSC

SEQ ID NO: 44 - protein, 17 aa, Artificial Sequence
  synthetic
CLTILYGYRWPLPSKLC

SEQ ID NO: 45 - protein, 29 aa, Artificial Sequence
  synthetic
CLYGYRWPLPSKLSCSDAFNWTVDSENRC

SEQ ID NO: 46 - protein, 29 aa, Artificial Sequence
  synthetic
CDSKVFKEGSSLLACSGEANTSDAFNWTC

SEQ ID NO: 47 - protein, 29 aa, Artificial Sequence
  synthetic
CVFKEGSSLLADDNCKESSNEDVIGALLC

SEQ ID NO: 48 - protein, 29 aa, Artificial Sequence
  synthetic
CLSEENTSLSSTTNCMDILSEENTSLSSC

SEQ ID NO: 49 - protein, 29 aa, Artificial Sequence
  synthetic
CLTILYGYRWPLPSCLYGYRWPLPSKLSC

SEQ ID NO: 50 - protein, 17 aa, Artificial Sequence
  synthetic
CLTILYGYRWPAASKLC

SEQ ID NO: 51 - protein, 29 aa, Artificial Sequence
  synthetic
CTRLYSNDFNSGEACKESSNEDVIGALLC

SEQ ID NO: 52 - protein, 29 aa, Artificial Sequence
  synthetic
CLYGYRWPLPSKLSCSGEANTSDAFNWTC

SEQ ID NO: 53 - protein, 29 aa, Artificial Sequence
  synthetic
CMDILSEENTSLSSCSKESSNEDVIGALC

SEQ ID NO: 54 - protein, 29 aa, Artificial Sequence
  synthetic
CSSLSLLHLQEKNWCMDILSEENTSLSSC

SEQ ID NO: 55 - protein, 29 aa, Artificial Sequence
  synthetic
CDSKVFKEGSSLLACSENRTNLSSEGSLC

SEQ ID NO: 56 - protein, 29 aa, Artificial Sequence
  synthetic
CVFKEGSSLLADDNCSDAFNWTVDSENRC

SEQ ID NO: 57 - protein, 29 aa, Artificial Sequence
  synthetic
CLQDDSKVFKEGSSCKESSNEDVIGALLC

SEQ ID NO: 58 - protein, 9 aa, Artificial Sequence
  synthetic
NFARKRIKN

SEQ ID NO: 59 - protein, 9 aa, Artificial Sequence
  synthetic
LNFARKRIK

SEQ ID NO: 60 - protein, 11 aa, Artificial Sequence
  synthetic
CNFARKRIKNC

SEQ ID NO: 61 - protein, 33 aa, Artificial Sequence
  synthetic
CSYLNFARKRIKNPEGCQNESYLNFARKRIKNC

SEQ ID NO: 62 - protein, 15 aa, Artificial Sequence
  synthetic
NESYLNFARKAAKNP

SEQ ID NO: 63 - protein, 15 aa, Artificial Sequence
  synthetic
QNESYLNFARKRIKN

SEQ ID NO: 64 - protein, 33 aa, Artificial Sequence
  synthetic
CVSEQKISEWGKIKESCQNESYLNFARKRIKNC

SEQ ID NO: 65 - protein, 33 aa, Artificial Sequence
  synthetic
CNFARKRIKNPEGGLYCQNESYLNFARKRIKNC

SEQ ID NO: 66 - protein, 33 aa, Artificial Sequence
  synthetic
CVRGQTAESLAVHNITCQNESYLNFARKRIKNC

SEQ ID NO: 67 - protein, 9 aa, Artificial Sequence
  synthetic
FARKRIKNP

SEQ ID NO: 68 - protein, 15 aa, Artificial Sequence
  synthetic
GDRQNESYLNAGRKR

SEQ ID NO: 69 - protein, 33 aa, Artificial Sequence
  synthetic
CQKISEWGKIKESPIPCQNESYLNFARKRIKNC

SEQ ID NO: 70 - protein, 33 aa, Artificial Sequence
  synthetic
CGDRQNESYLNFARKRCQNESYLNFARKRIKNC

SEQ ID NO: 71 - protein, 15 aa, Artificial Sequence
  synthetic
SYLNFARKRIAAPEG

SEQ ID NO: 72 - protein, 33 aa, Artificial Sequence
  synthetic
CEWSVNARVNNSDPYSCPYSVALSELGDRQNEC

SEQ ID NO: 73 - protein, 33 aa, Artificial Sequence
  synthetic
CHGAERIVRGQTAESLCQNESYLNFARKRIKNC

SEQ ID NO: 74 - protein, 33 aa, Artificial Sequence
  synthetic
CESLAVHNITVSEQKICQNESYLNFARKRIKNC

SEQ ID NO: 75 - protein, 33 aa, Artificial Sequence
  synthetic
CERIVRGQTAESLAVHCQNESYLNFARKRIKNC

SEQ ID NO: 76 - protein, 15 aa, Artificial Sequence
  synthetic
RQNESYLNFARKRIK

SEQ ID NO: 77 - protein, 15 aa, Artificial Sequence
  synthetic
NFARKRIKNPAAGLY

SEQ ID NO: 78 - protein, 15 aa, Artificial Sequence
  synthetic
DPYSVALSELAARQN

SEQ ID NO: 79 - protein, 33 aa, Artificial Sequence
  synthetic
CESLAVHNITVSEQKICSYLNFARKRIKNPEGC

SEQ ID NO: 80 - protein, 33 aa, Artificial Sequence
  synthetic
CSELGDRQNESYLNFACQNESYLNFARKRIKNC

SEQ ID NO: 81 - protein, 33 aa, Artificial Sequence
  synthetic
CNITVSEQKISEWGKICQNESYLNFARKRIKNC

SEQ ID NO: 82 - protein, 33 aa, Artificial Sequence
  synthetic
CHGAERIVRGQTAESLCSYLNFARKRIKNPEGC

SEQ ID NO: 83 - protein, 9 aa, Artificial Sequence
  synthetic
KISEWGKIK

SEQ ID NO: 84 - protein, 33 aa, Artificial Sequence
  synthetic
CVSEQKISEWGKIKESCEQKISEWGKIKESPIC

SEQ ID NO: 85 - protein, 33 aa, Artificial Sequence
  synthetic
CGDRQNESYLNFARKRCGDRQNESYLNFARKRC

SEQ ID NO: 86 - protein, 17 aa, Artificial Sequence
  synthetic
CNESYLNFARKAAKNPC

SEQ ID NO: 87 - protein, 11 aa, Artificial Sequence
  synthetic
CLNFARKRIKC

SEQ ID NO: 88 - protein, 15 aa, Artificial Sequence
  synthetic
QKISEWGKIKAAPIP

SEQ ID NO: 89 - protein, 33 aa, Artificial Sequence
  synthetic
CHGAERIVRGQTAESLCNFARKRIKNPEGGLYC

SEQ ID NO: 90 - protein, 17 aa, Artificial Sequence
  synthetic
CQNESYLNFARKRIKNC

SEQ ID NO: 91 - protein, 15 aa, Artificial Sequence
  synthetic
LNFARKRIKNAAGGL

SEQ ID NO: 92 - protein, 17 aa, Artificial Sequence
  synthetic
CLNFARKRIKNAAGGLC

SEQ ID NO: 93 - protein, 33 aa, Artificial Sequence
  synthetic
CQKISEWGKIKESPIPCTVSEQKISEWGKIKEC

SEQ ID NO: 94 - protein, 15 aa, Artificial Sequence
  synthetic
TVCEQKISEWGKIKE

SEQ ID NO: 95 - protein, 17 aa, Artificial Sequence
  synthetic
CRQNESYLNFARKRIKC

SEQ ID NO: 96 - protein, 15 aa, Artificial Sequence
  synthetic
NITVCEQKISAAGKI

SEQ ID NO: 97 - protein, 33 aa, Artificial Sequence
  synthetic
CNFARKRIKNPEGGLYCSYLNFARKRIKNPEGC

SEQ ID NO: 98 - protein, 33 aa, Artificial Sequence
  synthetic
CQKISEWGKIKESPIPCVSEQKISEWGKIKESC

SEQ ID NO: 99 - protein, 33 aa, Artificial Sequence
  synthetic
CNITVSEQKISEWGKICSYLNFARKRIKNPEGC

SEQ ID NO: 100 - protein, 33 aa, Artificial Sequence
  synthetic
CQTAESLAVHNITVSECQNESYLNFARKRIKNC

SEQ ID NO: 101 - protein, 33 aa, Artificial Sequence
  synthetic
CHGAERIVRGQTAESLCQKISEWGKIKESPIPC

SEQ ID NO: 102 - protein, 9 aa, Artificial Sequence
  synthetic
GKIKECPIP

SEQ ID NO: 103 - protein, 33 aa, Artificial Sequence
  synthetic
CEWSVNARVNNSDPYSCQNESYLNFARKRIKNC

SEQ ID NO: 104 - protein, 15 aa, Artificial Sequence
  synthetic
LGDRQNESYLNFARK

SEQ ID NO: 105 - protein, 17 aa, Artificial Sequence
  synthetic
CNITVSEQKISAAGKIC

SEQ ID NO: 106 - protein, 33 aa, Artificial Sequence
  synthetic
CNFARKRIKNPEGGLYCSLAVHNITVSEQKISC

SEQ ID NO: 107 - protein, 9 aa, Artificial Sequence
  synthetic
ESYLNFARK

SEQ ID NO: 108 - protein, 11 aa, Artificial Sequence
  synthetic
CKISEWGKIKC

SEQ ID NO: 109 - protein, 15 aa, Artificial Sequence
  synthetic
NESYLNFARKRIKNP

SEQ ID NO: 110 - protein, 33 aa, Artificial Sequence
  synthetic
CVALSELGDRQNESYLCQNESYLNFARKRIKNC

SEQ ID NO: 111 - protein, 33 aa, Artificial Sequence
  synthetic
CQNESYLNFARKRIKNCVSEQKISEWGKIKESC

SEQ ID NO: 112 - protein, 33 aa, Artificial Sequence
  synthetic
CVSEQKISEWGKIKESCGDRQNESYLNFARKRC

SEQ ID NO: 113 - protein, 15 aa, Artificial Sequence
  synthetic
QNESYLNFARAAIKN

SEQ ID NO: 114 - protein, 17 aa, Artificial Sequence
  synthetic
CSEQKISEWGKIKESPC

SEQ ID NO: 115 - protein, 33 aa, Artificial Sequence
  synthetic
CVSEQKISEWGKIKESCVSEQKISEWGKIKESC

SEQ ID NO: 116 - protein, 9 aa, Artificial Sequence
  synthetic
WGKIKECPI

SEQ ID NO: 117 - protein, 33 aa, Artificial Sequence
  synthetic
CNFARKRIKNPEGGLYCGDRQNESYLNFARKRC

SEQ ID NO: 118 - protein, 15 aa, Artificial Sequence
  synthetic
VNARVNNSDPAAVAL

SEQ ID NO: 119 - protein, 15 aa, Artificial Sequence
  synthetic
YLNFARKRIKAAEGG

SEQ ID NO: 120 - protein, 15 aa, Artificial Sequence
  synthetic
GDRQNESYLNFARKR

SEQ ID NO: 121 - protein, 15 aa, Artificial Sequence
  synthetic
WCVNARVNNSDPYSV

SEQ ID NO: 122 - protein, 33 aa, Artificial Sequence
  synthetic
CSYLNFARKRIKNPEGCITVSEQKISEWGKIKC

SEQ ID NO: 123 - protein, 33 aa, Artificial Sequence
  synthetic
CAVHNITVSEQKISEWCVSEQKISEWGKIKESC

SEQ ID NO: 124 - protein, 33 aa, Artificial Sequence
  synthetic
CPYSVALSELGDRQNECITVSEQKISEWGKIKC

SEQ ID NO: 125 - protein, 33 aa, Artificial Sequence
  synthetic
CSYLNFARKRIKNPEGCGDRQNESYLNFARKRC

SEQ ID NO: 126 - protein, 33 aa, Artificial Sequence
  synthetic
CAVHNITVSEQKISEWCQNESYLNFARKRIKNC

SEQ ID NO: 127 - protein, 15 aa, Artificial Sequence
  synthetic
LGDRQNESYLAAARK

SEQ ID NO: 128 - protein, 33 aa, Artificial Sequence
  synthetic
CVNARVNNSDPYSVALCVSEQKISEWGKIKESC

SEQ ID NO: 129 - protein, 33 aa, Artificial Sequence
  synthetic
CFNVEWSVNARVNNSDCGDRQNESYLNFARKRC

SEQ ID NO: 130 - protein, 33 aa, Artificial Sequence
  synthetic
CNSDPYSVALSELGDRCVSEQKISEWGKIKESC

SEQ ID NO: 131 - protein, 33 aa, Artificial Sequence
  synthetic
CGDRQNESYLNFARKRCSYLNFARKRIKNPEGC

SEQ ID NO: 132 - protein, 15 aa, Artificial Sequence
  synthetic
DPYSVALSELGDRQN

SEQ ID NO: 133 - protein, 33 aa, Artificial Sequence
  synthetic
CAVHNITVSEQKISEWCSYLNFARKRIKNPEGC

SEQ ID NO: 134 - protein, 33 aa, Artificial Sequence
  synthetic
CVRGQTAESLAVHNITCITVSEQKISEWGKIKC

SEQ ID NO: 135 - protein, 33 aa, Artificial Sequence
  synthetic
CQNESYLNFARKRIKNCSYLNFARKRIKNPEGC

SEQ ID NO: 136 - protein, 33 aa, Artificial Sequence
  synthetic
CESLAVHNITVSEQKICGDRQNESYLNFARKRC

SEQ ID NO: 137 - protein, 33 aa, Artificial Sequence
  synthetic
CRVNNSDPYSVALSELCQNESYLNFARKRIKNC

SEQ ID NO: 138 - protein, 33 aa, Artificial Sequence
  synthetic
CSYLNFARKRIKNPEGCNFARKRIKNPEGGLYC

SEQ ID NO: 139 - protein, 33 aa, Artificial Sequence
  synthetic
CQTAESLAVHNITVSECVSEQKISEWGKIKESC

SEQ ID NO: 140 - protein, 9 aa, Artificial Sequence
  synthetic
YLNFARKRI

SEQ ID NO: 141 - protein, 33 aa, Artificial Sequence
  synthetic
CFNVEWSVNARVNNSDCVSEQKISEWGKIKESC

SEQ ID NO: 142 - protein, 33 aa, Artificial Sequence
  synthetic
CVSEQKISEWGKIKESCTVSEQKISEWGKIKEC

SEQ ID NO: 143 - protein, 33 aa, Artificial Sequence
  synthetic
CNSDPYSVALSELGDRCITVSEQKISEWGKIKC

SEQ ID NO: 144 - protein, 33 aa, Artificial Sequence
  synthetic
CNITVSEQKISEWGKICGDRQNESYLNFARKRC

SEQ ID NO: 145 - protein, 17 aa, Artificial Sequence
  synthetic
CLGDRQNESYLAAARKC

SEQ ID NO: 146 - protein, 9 aa, Artificial Sequence
  synthetic
QKISEWGKI

SEQ ID NO: 147 - protein, 17 aa, Artificial Sequence
  synthetic
CITVSEQKISEAAKIKC

SEQ ID NO: 148 - protein, 33 aa, Artificial Sequence
  synthetic
CVRGQTAESLAVHNITCVHNITVSEQKISEWGC

SEQ ID NO: 149 - protein, 33 aa, Artificial Sequence
  synthetic
CQKISEWGKIKESPIPCVHNITVSEQKISEWGC

SEQ ID NO: 150 - protein, 33 aa, Artificial Sequence
  synthetic
CQNESYLNFARKRIKNCNFARKRIKNPEGGLYC

SEQ ID NO: 151 - protein, 33 aa, Artificial Sequence
  synthetic
CRVNNSDPYSVALSELCVSEQKISEWGKIKESC

SEQ ID NO: 152 - protein, 33 aa, Artificial Sequence
  synthetic
CGDRQNESYLNFARKRCVSEQKISEWGKIKESC

SEQ ID NO: 153 - protein, 17 aa, Artificial Sequence
  synthetic
CQKISEWGKIKAAPIPC

SEQ ID NO: 154 - protein, 33 aa, Artificial Sequence
  synthetic
CVNARVNNSDPYSVALCTVSEQKISEWGKIKEC

SEQ ID NO: 155 - protein, 33 aa, Artificial Sequence
  synthetic
CEWSVNARVNNSDPYSCVSEQKISEWGKIKESC

SEQ ID NO: 156 - protein, 33 aa, Artificial Sequence
  synthetic
CVRGQTAESLAVHNITCSLAVHNITVSEQKISC

SEQ ID NO: 157 - protein, 10 aa, Artificial Sequence
  synthetic
DDSKVFKEGS

SEQ ID NO: 158 - protein, 12 aa, Artificial Sequence
  synthetic
LYGYRWPLPSKL

SEQ ID NO: 159 - DNA, 20 bp, Artificial Sequence
  synthetic
ttaacagcacgctgatcctg

SEQ ID NO: 160 - DNA, 20 bp, Artificial Sequence
  synthetic
cactccagtgagaccagcaa

SEQ ID NO: 161 - DNA, 25 bp, Artificial Sequence
  synthetic
ggagtttcaagatgcgtggaaacta

SEQ ID NO: 162 - DNA, 24 bp, Artificial Sequence
  synthetic
gccagactcagagttggagatgct

SEQ ID NO: 163 - DNA, 20 bp, Artificial Sequence
  synthetic
ccagggcagtacatcttggt

SEQ ID NO: 164 - DNA, 20 bp, Artificial Sequence
  synthetic
ccgtgtttccagggagagta

SEQ ID NO: 165 - DNA, 20 bp, Artificial Sequence
  synthetic
gcttacctccgaggatcaca

SEQ ID NO: 166 - DNA, 19 bp, Artificial Sequence
  synthetic
cgggagggtgggtatctaa

SEQ ID NO: 167 - DNA, 24 bp, Artificial Sequence
  synthetic
atcaagcggccccctttttttcac

SEQ ID NO: 168 - DNA, 24 bp, Artificial Sequence
  synthetic
ctcattgtcacactcctcgacagc

SEQ ID NO: 169 - DNA, 20 bp, Artificial Sequence
  synthetic
tcatcatggcagtgtcccta

SEQ ID NO: 170 - DNA, 20 bp, Artificial Sequence
  synthetic
tgagggaggaagctgaaaga

SEQ ID NO: 171 - DNA, 20 bp, Artificial Sequence
  synthetic
tcaccctgaagtaccccatc

SEQ ID NO: 172 - DNA, 18 bp, Artificial Sequence
  synthetic
ggctggaagagtgcctca

SEQ ID NO: 173 - protein, 10 aa, Artificial Sequence
  synthetic
TWYAHNCRLQ